European Patent Application EP 4 148 129 A1, published March 15, 2023. Title: Directed evolution method based on primary and secondary replicons of geminivirus. Applicant: Suzhou Qi Biodesign biotechnology Company Limited. The sequence listing filed with the application follows.

SEQUENCE LISTING (6 sequences)

SEQ ID NO: 1 - DNA, 409 bp, Wheat dwarf virus
  WDV-LIR
ggtagtgaacagaagtccggcaggtccttagcgaaaaaacggggtgtgccagaaaactctatcctctaccctgcgtggaggtgtgaattctgcacactgcaaatgcaatgtgtccaatgctttatatagggcaggttttggcgggagaacagggccctagtgttcccacggtagcgtagcgaatcgtgtgggccctgttcggtgtgcggtcggggggcctccacgcgggttataatattaccccgcgtggtggcccccgacgcgcactcggcttttcgtgagtgcgcggaggcttttggaccacatcttttctgatcactttcgtggaagatgttgatttatcacacttttgacggggaaatctgtgccatgccttagcttataaggaagtgcgtggtagcccatctcg

SEQ ID NO: 2 - DNA, 171 bp, Wheat dwarf virus
  WDV-SIR
taaaataatattttatttatctcatgtcattcgattacagaggctcggctacgagcaaagacaaaccaaatataacaaacaacaacccttacacaatgacatcggaaaacgaaatacaacaccctgagatattacatttatagaaactgtacgccgtccgcgctaggacag

SEQ ID NO: 3 - protein, 351 aa, Wheat dwarf virus
  WDV-Rep
MASSSAPRFRVYSKYLFLTYPQCTLEPQYALDSLRTLLNKYEPLYIAAVRELHEDGSPHLHVLVQNKLRASITNPNALNLRMDTSPFSIFHPNIQAAKDCNQVRDYITKEVDSDVNTAEWGTFVAVSTPGRKDRDADMKQIIESSSSREEFLSMVCNRFPFEWSIRLKDFEYTARHLFPDPVATYTPEFPTESLICHETIESWKNEHLYSESPGRHKSIYICGPTRTGKTSWARSLGTHNYYNSLVDFTTYDVNAKYNIIDDIPFKFTPNWKCFVGAQRDFTVNPKYGKRKVIRGGIPCIILVNPDEDWLKDMTPEQSDYMYSNTVVHYMYEGETFINYSFASGEDVTASQ

SEQ ID NO: 4 - protein, 351 aa, Artificial Sequence
  WDV-Rep Y20C
MASSSAPRFRVYSKYLFLTCPQCTLEPQYALDSLRTLLNKYEPLYIAAVRELHEDGSPHLHVLVQNKLRASITNPNALNLRMDTSPFSIFHPNIQAAKDCNQVRDYITKEVDSDVNTAEWGTFVAVSTPGRKDRDADMKQIIESSSSREEFLSMVCNRFPFEWSIRLKDFEYTARHLFPDPVATYTPEFPTESLICHETIESWKNEHLYSESPGRHKSIYICGPTRTGKTSWARSLGTHNYYNSLVDFTTYDVNAKYNIIDDIPFKFTPNWKCFVGAQRDFTVNPKYGKRKVIRGGIPCIILVNPDEDWLKDMTPEQSDYMYSNTVVHYMYEGETFINYSFASGEDVTASQ

SEQ ID NO: 5 - protein, 264 aa, Wheat dwarf virus
  WDV-RepA
MASSSAPRFRVYSKYLFLTYPQCTLEPQYALDSLRTLLNKYEPLYIAAVRELHEDGSPHLHVLVQNKLRASITNPNALNLRMDTSPFSIFHPNIQAAKDCNQVRDYITKEVDSDVNTAEWGTFVAVSTPGRKDRDADMKQIIESSSSREEFLSMVCNRFPFEWSIRLKDFEYTARHLFPDPVATYTPEFPTESLICHETIESWKNEHLYSVSLESYILCTSTPADQAQSDLEWMDDYSRSHRGGISPSTSAGQPEQERLPGQGL

SEQ ID NO: 6 - protein, 264 aa, Artificial Sequence
  WDV-RepA Y20C
MASSSAPRFRVYSKYLFLTCPQCTLEPQYALDSLRTLLNKYEPLYIAAVRELHEDGSPHLHVLVQNKLRASITNPNALNLRMDTSPFSIFHPNIQAAKDCNQVRDYITKEVDSDVNTAEWGTFVAVSTPGRKDRDADMKQIIESSSSREEFLSMVCNRFPFEWSIRLKDFEYTARHLFPDPVATYTPEFPTESLICHETIESWKNEHLYSVSLESYILCTSTPADQAQSDLEWMDDYSRSHRGGISPSTSAGQPEQERLPGQGL